European Patent Specification EP 4 127 711 B1, published December 24, 2025. Title: METHOD. Applicant: OXFORD NANOPORE TECHNOLOGIES LIMITED. The sequence listing filed with the application follows.

SEQUENCE LISTING (8 sequences)

SEQ ID NO: 1 - protein, 485 aa, Escherichia coli
MMNDGKQQSTFLFHDYETFGTHPALDRPAQFAAIRTDSEFNVIGEPEVFYCKPADDYLPQPGAVLITGITPQEARAKGENEAAFAARIHSLFTVPKTCILGYNNVRFDDEVTRNIFYRNFYDPYAWSWQHDNSRWDLLDVMRACYALRPEGINWPENDDGLPSFRLEHLTKANGIEHSNAHDAMADVYATIAMAKLVKTRQPRLFDYLFTHRNKHKLMALIDVPQMKPLVHVSGMFGAWRGNTSWVAPLAWHPENRNAVIMVDLAGDISPLLELDSDTLRERLYTAKTDLGDNAAVPVKLVHINKCPVLAQANTLRPEDADRLGINRQHCLDNLKILRENPQVREKVVAIFAEAEPFTPSDNVDAQLYNGFFSDADRAAMKIVLETEPRNLPALDITFVDKRIEKLLFNYRARNFPGTLDYAEQQRWLEHRRQVFTPEFLQGYADELQMLVQQYADDKEKVALLKALWQYAEEIVSGSGHHHHHH

SEQ ID NO: 2 - protein, 268 aa, Escherichia coli
MKFVSFNINGLRARPHQLEAIVEKHQPDVIGLQETKVHDDMFPLEEVAKLGYNVFYHGQKGHYGVALLTKETPIAVRRGFPGDDEEAQRRIIMAEIPSLLGNVTVINGYFPQGESRDHPIKFPAKAQFYQNLQNYLETELKRDNPVLIMGDMNISPTDLDIGIGEENRKRWLRTGKCSFLPEEREWMDRLMSWGLVDTFRHANPQTADRFSWFDYRSKGFDDNRGLRIDLLLASQPLAECCVETGIDYEIRSMEKPSDHAPVWATFRR

SEQ ID NO: 3 - protein, 425 aa, Thermus thermophilus
MFRRKEDLDPPLALLPLKGLREAAALLEEALRQGKRIRVHGDYDADGLTGTAILVRGLAALGADVHPFIPHRLEEGYGVLMERVPEHLEASDLFLTVDCGITNHAELRELLENGVEVIVTDHHTPGKTPPPGLVVHPALTPDLKEKPTGAGVAFLLLWALHERLGLPPPLEYADLAAVGTIADVAPLWGWNRALVKEGLARIPASSWVGLRLLAEAVGYTGKAVEVAFRIAPRINAASRLGEAEKALRLLLTDDAAEAQALVGELHRLNARRQTLEEAMLRKLLPQADPEAKAIVLLDPEGHPGVMGIVASRILEATLRPVFLVAQGKGTVRSLAPISAVEALRSAEDLLLRYGGHKEAAGFAMDEALFPAFKARVEAYAARFPDPVREVALLDLLPEPGLLPQVFRELALLEPYGEGNPEPLFL

SEQ ID NO: 4 - protein, 226 aa, Bacteriophage lambda
MTPDIILQRTGIDVRAVEQGDDAWHKLRLGVITASEVHNVIAKPRSGKKWPDMKMSYFHTLLAEVCTGVAPEVNAKALAWGKQYENDARTLFEFTSGVNVTESPIIYRDESMRTACSPDGLCSDGNGLELKCPFTSRDFMKFRLGGFEAIKSAYMAQVQYSMWVTRKNAWYFANYDPRMKREGLHYVVIERDEKYMASFDEIVPEFIEKMDEALAEIGFVFGEQWR

SEQ ID NO: 5 - protein, 608 aa, Bacillus subtilis phage Phi 29
MKHMPRKMYSCAFETTTKVEDCRVWAYGYMNIEDHSEYKIGNSLDEFMAWVLKVQADLYFHNLKFDGAFIINWLERNGFKWSADGLPNTYNTIISRMGQWYMIDICLGYKGKRKIHTVIYDSLKKLPFPVKKIAKDFKLTVLKGDIDYHKERPVGYKITPEEYAYIKNDIQIIAEALLIQFKQGLDRMTAGSDSLKGFKDIITTKKFKKVFPTLSLGLDKEVRYAYRGGFTWLNDRFKEKEIGEGMVFDVNSLYPAQMYSRLLPYGEPIVFEGKYVWDEDYPLHIQHIRCEFELKEGYIPTIQIKRSRFYKGNEYLKSSGGEIADLWLSNVDLELMKEHYDLYNVEYISGLKFKATTGLFKDFIDKWTYIKTTSEGAIKQLAKLMLNSLYGKFASNPDVTGKVPYLKENGALGFRLGEEETKDPVYTPMGVFITAWARYTTITAAQACYDRIIYCDTDSIHLTGTEIPDVIKDIVDPKKLGYWAHESTFKRAKYLRQKTYIQDIYMKEVDGKLVEGSPDDYTDIKFSVKCAGMTDKIKKEVTFENFKVGFSRKMKPKPVQVPGGVVLVDDTFTIKSGGSAWSHPQFEKGGGSGGGSGGSAWSHPQFEK

SEQ ID NO: 6 - protein, 970 aa, Citromicrobium bathyomarinum
MLSVANVRSPSAAASYFASDNYYASADADRSGQWIGDGAKRLGLEGKVEARAFDALLRGELPDGSSVGNPGQAHRPGTDLTFSVPKSWSLLALVGKDERIIAAYREAVVEALHWAEKNAAETRVVEKGMVVTQATGNLAIGLFQHDTNRNQEPNLHFHAVIANVTQGKDGKWRTLKNDRLWQLNTTLNSIAMARFRVAVEKLGYEPGPVLKHGNFEARGISREQVMAFSTRRKEVLEARRGPGLDAGRIAALDTRASKEGIEDRATLSKQWSEAAQSIGLDLKPLVDRARTKALGQGMEATRIGSLVERGRAWLSRFAAHVRGDPADPLVPPSVLKQDRQTIAAAQAVASAVRHLSQREAAFERTALYKAALDFGLPTTIADVEKRTRALVRSGDLIAGKGEHKGWLASRDAVVTEQRILSEVAAGKGDSSPAITPQKAAASVQAAALTGQGFRLNEGQLAAARLILISKDRTIAVQGIAGAGKSSVLKPVAEVLRDEGHPVIGLAIQNTLVQMLERDTGIGSQTLARFLGGWNKLLDDPGNVALRAEAQASLKDHVLVLDEASMVSNEDKEKLVRLANLAGVHRLVLIGDRKQLGAVDAGKPFALLQRAGIARAEMATNLRARDPVVREAQAAAQAGDVRKALRHLKSHTVEARGDGAQVAAETWLALDKETRARTSIYASGRAIRSAVNAAVQQGLLASREIGPAKMKLEVLDRVNTTREELRHLPAYRAGRVLEVSRKQQALGLFIGEYRVIGQDRKGKLVEVEDKRGKRFRFDPARIRAGKGDDNLTLLEPRKLEIHEGDRIRWTRNDHRRGLFNADQARVVEIANGKVTFETSKGDLVELKKDDPMLKRIDLAYALNVHMAQGLTSDRGIAVMDSRERNLSNQKTFLVTVTRLRDHLTLVVDSADKLGAAVARNKGEKASAIEVTGSVKPTATKGSGVDQPKSVEANKAEKELTRSKSKTLDFGI

SEQ ID NO: 7 - protein, 760 aa, Methanococcoides burtonii
MMIRELDIPRDIIGFYEDSGIKELYPPQAEAIEMGLLEKKNLLAAIPTASGKTLLAELAMIKAIREGGKALYIVPLRALASEKFERFKELAPFGIKVGISTGDLDSRADWLGVNDIIVATSEKTDSLLRNGTSWMDEITTVVVDEIHLLDSKNRGPTLEVTITKLMRLNPDVQVVALSATVGNAREMADWLGAALVLSEWRPTDLHEGVLFGDAINFPGSQKKIDRLEKDDAVNLVLDTIKAEGQCLVFESSRRNCAGFAKTASSKVAKILDNDIMIKLAGIAEEVESTGETDTAIVLANCIRKGVAFHHAGLNSNHRKLVENGFRQNLIKVISSTPTLAAGLNLPARRVIIRSYRRFDSNFGMQPIPVLEYKQMAGRAGRPHLDPYGESVLLAKTYDEFAQLMENYVEADAEDIWSKLGTENALRTHVLSTIVNGFASTRQELFDFFGATFFAYQQDKWMLEEVINDCLEFLIDKAMVSETEDIEDASKLFLRGTRLGSLVSMLYIDPLSGSKIVDGFKDIGKSTGGNMGSLEDDKGDDITVTDMTLLHLVCSTPDMRQLYLRNTDYTIVNEYIVAHSDEFHEIPDKLKETDYEWFMGEVKTAMLLEEWVTEVSAEDITRHFNVGEGDIHALADTSEWLMHAAAKLAELLGVEYSSHAYSLEKRIRYGSGLDLMELVGIRGVGRVRARKLYNAGFVSVAKLKGADISVLSKLVGPKVAYNILSGIGVRVNDKHFNSAPISSNTLDTLLDKNQKTFNDFQ

SEQ ID NO: 8 - protein, 439 aa, Enterobacteria phage T4
MTFDDLTEGQKNAFNIVMKAIKEKKHHVTINGPAGTGKTTLTKFIIEALISTGETGIILAAPTHAAKKILSKLSGKEASTIHSILKINPVTYEENVLFEQKEVPDLAKCRVLICDEVSMYDRKLFKILLSTIPPWCTIIGIGDNKQIRPVDPGENTAYISPFFTHKDFYQCELTEVKRSNAPIIDVATDVRNGKWIYDKVVDGHGVRGFTGDTALRDFMVNYFSIVKSLDDLFENRVMAFTNKSVDKLNSIIRKKIFETDKDFIVGEIIVMQEPLFKTYKIDGKPVSEIIFNNGQLVRIIEAEYTSTFVKARGVPGEYLIRHWDLTVETYGDDEYYREKIKIISSDEELYKFNLFLGKTAETYKNWNKGGKAPWSDFWDAKSQFSKVKALPASTFHKAQGMSVDRAFIYTPCIHYADVELAQQLLYVGVTRGRYDVFYV